European Patent Specification EP 3 156 066 B1, published April 26, 2023. Title: Composition for Treating Diabetes Comprising Long-acting Insulin Analogue Conjugate and Long-acting Insulinotropic Peptide Conjugate. Applicant: HANMI PHARM. CO., LTD. The sequence listing filed with the application follows.

SEQUENCE LISTING (41 sequences)

SEQ ID NO: 1 - DNA, 39 bp, Artificial Sequence
  Primer
gggtccctgcagaagcgtgcgattgtggaacaatgctgt

SEQ ID NO: 2 - DNA, 39 bp, Artificial Sequence
  Primer
acagcattgttccacaatcgcacgcttctgcagggaccc

SEQ ID NO: 3 - DNA, 39 bp, Artificial Sequence
  Primer
tccctgcagaagcgtggcgcggtggaacaatgctgtacc

SEQ ID NO: 4 - DNA, 39 bp, Artificial Sequence
  Primer
ggtacagcattgttccaccgcgccacgcttctgcaggga

SEQ ID NO: 5 - DNA, 36 bp, Artificial Sequence
  Primer
ctctaccagctggaaaacgcgtgtaactgaggatcc

SEQ ID NO: 6 - DNA, 36 bp, Artificial Sequence
  Primer
ggatcctcagttacacgcgttttccagctggtagag

SEQ ID NO: 7 - DNA, 39 bp, Artificial Sequence
  Primer
gttaaccaacacttgtgtgcgtcacacctggtggaagct

SEQ ID NO: 8 - DNA, 39 bp, Artificial Sequence
  Primer
agcttccaccaggtgtgacgcacacaagtgttggttaac

SEQ ID NO: 9 - DNA, 39 bp, Artificial Sequence
  Primer
ctagtgtgcggggaacgagcgttcttctacacacccaag

SEQ ID NO: 10 - DNA, 39 bp, Artificial Sequence
  Primer
cttgggtgtgtagaagaacgctcgttccccgcacactag

SEQ ID NO: 11 - DNA, 39 bp, Artificial Sequence
  Primer
gtgtgcggggaacgaggcgcgttctacacacccaagacc

SEQ ID NO: 12 - DNA, 39 bp, Artificial Sequence
  Primer
ggtcttgggtgtgtagaacgcgcctcgttccccgcacac

SEQ ID NO: 13 - DNA, 39 bp, Artificial Sequence
  Primer
tgcggggaacgaggcttcgcgtacacacccaagacccgc

SEQ ID NO: 14 - DNA, 39 bp, Artificial Sequence
  Primer
gcgggtcttgggtgtgtacgcgaagcctcgttccccgca

SEQ ID NO: 15 - DNA, 37 bp, Artificial Sequence
  Primer
ccagcatctgctccctcgaacagctggagaactactg

SEQ ID NO: 16 - DNA, 37 bp, Artificial Sequence
  Primer
cagtagttctccagctgttcgagggagcagatgctgg

SEQ ID NO: 17 - DNA, 34 bp, Artificial Sequence
  Primer
cagcatctgctccctcaaccagctggagaactac

SEQ ID NO: 18 - DNA, 34 bp, Artificial Sequence
  Primer
gtagttctccagctggttgagggagcagatgctg

SEQ ID NO: 19 - DNA, 258 bp, Artificial Sequence
  Analog 1
ttcgttaaccaacacttgtgtggctcacacctggtggaagctctctacctagtgtgcggggaacgaggcttcttctacacacccaagacccgccgggaggcagaggacctgcaggtggggcaggtggagctgggcgggggccctggtgcaggcagcctgcagcccttggccctggaggggtccctgcagaagcgtgcgattgtggaacaatgctgtaccagcatctgctccctctaccagctggagaactactgcaac

SEQ ID NO: 20 - protein, 86 aa, Artificial Sequence
  Analog 1
FVNQHLCGSHLVEALYLVCGERGFFYTPKTRREAEDLQVGQVELGGGPGAGSLQPLALEGSLQKRAIVEQCCTSICSLYQLENYCN

SEQ ID NO: 21 - DNA, 258 bp, Artificial Sequence
  Analog 2
ttcgttaaccaacacttgtgtggctcacacctggtggaagctctctacctagtgtgcggggaacgaggcttcttctacacacccaagacccgccgggaggcagaggacctgcaggtggggcaggtggagctgggcgggggccctggtgcaggcagcctgcagcccttggccctggaggggtccctgcagaagcgtggcgcggtggaacaatgctgtaccagcatctgctccctctaccagctggagaactactgcaac

SEQ ID NO: 22 - protein, 86 aa, Artificial Sequence
  Analog 2
FVNQHLCGSHLVEALYLVCGERGFFYTPKTRREAEDLQVGQVELGGGPGAGSLQPLALEGSLQKRGAVEQCCTSICSLYQLENYCN

SEQ ID NO: 23 - DNA, 258 bp, Artificial Sequence
  Analog 3
ttcgttaaccaacacttgtgtggctcacacctggtggaagctctctacctagtgtgcggggaacgaggcttcttctacacacccaagacccgccgggaggcagaggacctgcaggtggggcaggtggagctgggcgggggccctggtgcaggcagcctgcagcccttggccctggaggggtccctgcagaagcgtggcattgtggaacaatgctgtaccagcatctgctccctctaccagctggagaacgcgtgcaac

SEQ ID NO: 24 - protein, 86 aa, Artificial Sequence
  Analog 3
FVNQHLCGSHLVEALYLVCGERGFFYTPKTRREAEDLQVGQVELGGGPGAGSLQPLALEGSLQKRGIVEQCCTSICSLYQLENACN

SEQ ID NO: 25 - DNA, 258 bp, Artificial Sequence
  Analog 4
ttcgttaaccaacacttgtgtgcgtcacacctggtggaagctctctacctagtgtgcggggaacgaggcttcttctacacacccaagacccgccgggaggcagaggacctgcaggtggggcaggtggagctgggcgggggccctggtgcaggcagcctgcagcccttggccctggaggggtccctgcagaagcgtggcattgtggaacaatgctgtaccagcatctgctccctctaccagctggagaactactgcaac

SEQ ID NO: 26 - protein, 86 aa, Artificial Sequence
  Analog 4
FVNQHLCASHLVEALYLVCGERGFFYTPKTRREAEDLQVGQVELGGGPGAGSLQPLALEGSLQKRGIVEQCCTSICSLYQLENYCN

SEQ ID NO: 27 - DNA, 258 bp, Artificial Sequence
  Analog 5
ttcgttaaccaacacttgtgtggctcacacctggtggaagctctctacctagtgtgcggggaacgagcgttcttctacacacccaagacccgccgggaggcagaggacctgcaggtggggcaggtggagctgggcgggggccctggtgcaggcagcctgcagcccttggccctggaggggtccctgcagaagcgtggcattgtggaacaatgctgtaccagcatctgctccctctaccagctggagaactactgcaac

SEQ ID NO: 28 - protein, 86 aa, Artificial Sequence
  Analog 5
FVNQHLCGSHLVEALYLVCGERAFFYTPKTRREAEDLQVGQVELGGGPGAGSLQPLALEGSLQKRGIVEQCCTSICSLYQLENYCN

SEQ ID NO: 29 - DNA, 258 bp, Artificial Sequence
  Analog 6
ttcgttaaccaacacttgtgtggctcacacctggtggaagctctctacctagtgtgcggggaacgaggcgcgttctacacacccaagacccgccgggaggcagaggacctgcaggtggggcaggtggagctgggcgggggccctggtgcaggcagcctgcagcccttggccctggaggggtccctgcagaagcgtggcattgtggaacaatgctgtaccagcatctgctccctctaccagctggagaactactgcaac

SEQ ID NO: 30 - protein, 86 aa, Artificial Sequence
  Analog 6
FVNQHLCGSHLVEALYLVCGERGAFYTPKTRREAEDLQVGQVELGGGPGAGSLQPLALEGSLQKRGIVEQCCTSICSLYQLENYCN

SEQ ID NO: 31 - DNA, 258 bp, Artificial Sequence
  Analog 7
ttcgttaaccaacacttgtgtggctcacacctggtggaagctctctacctagtgtgcggggaacgaggcttcgcgtacacacccaagacccgccgggaggcagaggacctgcaggtggggcaggtggagctgggcgggggccctggtgcaggcagcctgcagcccttggccctggaggggtccctgcagaagcgtggcattgtggaacaatgctgtaccagcatctgctccctctaccagctggagaactactgcaac

SEQ ID NO: 32 - protein, 86 aa, Artificial Sequence
  Analog 7
FVNQHLCGSHLVEALYLVCGERGFAYTPKTRREAEDLQVGQVELGGGPGAGSLQPLALEGSLQKRGIVEQCCTSICSLYQLENYCN

SEQ ID NO: 33 - DNA, 261 bp, Artificial Sequence
  Analog 8
ttcgttaaccaacacttgtgtggctcacacctggtggaagctctctacctagtgtgcggggaacgaggcttcttctacacacccaagacccgccgggaggcagaggacctgcaggtggggcaggtggagctgggcgggggccctggtgcaggcagcctgcagcccttggccctggaggggtccctgcagaagcgtggcattgtggaacaatgctgtaccagcatctgctccctcgaacagctggagaactactgcaactga

SEQ ID NO: 34 - protein, 86 aa, Artificial Sequence
  Analog 8
FVNQHLCGSHLVEALYLVCGERGFFYTPKTRREAEDLQVGQVELGGGPGAGSLQPLALEGSLQKRGIVEQCCTSICSLEQLENYCN

SEQ ID NO: 35 - DNA, 261 bp, Artificial Sequence
  Analog 9
ttcgttaaccaacacttgtgtggctcacacctggtggaagctctctacctagtgtgcggggaacgaggcttcttctacacacccaagacccgccgggaggcagaggacctgcaggtggggcaggtggagctgggcgggggccctggtgcaggcagcctgcagcccttggccctggaggggtccctgcagaagcgtggcattgtggaacaatgctgtaccagcatctgctccctcaaccagctggagaactactgcaactga

SEQ ID NO: 36 - protein, 86 aa, Artificial Sequence
  Analog 9
FVNQHLCGSHLVEALYLVCGERGFFYTPKTRREAEDLQVGQVELGGGPGAGSLQPLALEGSLQKRGIVEQCCTSICSLNQLENYCN

SEQ ID NO: 37 - protein, 21 aa, Artificial Sequence
  A chain of insulin
GIVEQCCTSICSLYQLENYCN

SEQ ID NO: 38 - protein, 30 aa, Artificial Sequence
  B chain of insulin
FVNQHLCGSHLVEALYLVCGERGFFYTPKT

SEQ ID NO: 39 - protein, 31 aa, Artificial Sequence
  GLP-1(7-37)
HAEGTFTSDVSSYLEGQAAKEFIAWLVKGRG

SEQ ID NO: 40 - protein, 39 aa, Artificial Sequence
  exendin-3
HSDGTFTSDLSKQMEEEAVRLFIEWLKNGGPSSGAPPPS

SEQ ID NO: 41 - protein, 39 aa, Artificial Sequence
  exendin-4
HGEGTFTSDLSKQMEEEAVRLFIEWLKNGGPSSGAPPPS